European Patent Specification EP 3 152 323 B1, published October 23, 2024. Title: Optimization of DNA amplification reactions. Applicant: Qiagen GmbH. The sequence listing filed with the application follows.

SEQUENCE LISTING (4 sequences)

SEQ ID NO: 1 - DNA, 21 bp, Artificial sequence
  TNF alpha primer
ggtttcgaagtggtggtcttg

SEQ ID NO: 2 - DNA, 20 bp, Artificial sequence
  TNF alpha primer
cctgccccaatccctttatt

SEQ ID NO: 3 - DNA, 20 bp, Artificial sequence
  IL1R2 primer
cgggtaggcgctctctatgt

SEQ ID NO: 4 - DNA, 23 bp, Artificial sequence
  IL1R2 primer
aagactgacaatcccgtgtaagg